European Patent Application EP 4 353 824 A1, published April 17, 2024. Title: CONSTRUCT FOR INDUCING SILENCING IN PLANTS AND METHOD FOR PROTECTING THEM AGAINST TOMATO SPOTTED WILT VIRUS. Applicant: UNIVERSIDADE DE ÉVORA. The sequence listing filed with the application follows.

SEQUENCE LISTING (3 sequences)

SEQ ID NO: 1 - DNA, 3679 bp, Olive mild mosaic virus
  source 1..3679: mol_type = genomic DNA
agtatacataccaagtatacggaataggtgtgaacccttgctcagctaaagaggataaaatggagctcactaaccactgcaagcaaactgctgctgaaggatttgtaagctttctgaactggctttgtaacccatggagacgacaacgaacagtcaacgctgctgttaagttccaacaggctctcctctcaatagaggatactgaacacttcgaggacatcaacgaatgcctcgaggagtctgctggagcccaatcacagcgaactaaggttgtcgccgaaggggcatattctcccgtcaaaaccaatcgtacccgccgagtccgcaagcagaagaaggccaagtttgtcaagtacttggtcaatgaggctcgtgccgagtttggtctacccaaagccactgaggccaatcgacttatggtacaacacttcttgctcagaacgtgtaaggaatggggtgtggtcacctcccaatgtcataacaacgttgcacttgcgttaaacctagtgttcatcccaactgaagatgacctgctgtcccgagcactgatgaacacttacgccacgcgagctgctgtgaatggaatgaccaacacccaaggggaggggtggtggaacaaccgacttgggattggatcccaggttggactggccttccgggccaaataggggtgcctagagaggaggccagggttctccacgtccgtttcgcgtggagagcaccctgatctggtggtcaaaccatcaggacaccccgagaaacagcgccagttgctgcgctatagtggaattggcggccatttactaattggcatccacaacaactctctctccaatttgcgccggggcttaatggaaagagtattctacgtcgagggacccaatgggctccaagacgccccgaaacccgacaagggagccttcaactcccttgctaagttcagagatctctatacaaagaatagctggcgtcattcccctgtaaccaatgagcaatttttgatgaattactcgggcaggaagctaactatttacaaggatgcggtcgacagtttgtcgcgtcaaccgcttagcctaagagatgctcggctgaagacattcgttaaggcggaaaaattgaatctgagtaagaaaccagatccagcaccgagggtcattcagcctcggtcgccccgctataacgtatgtttgggtcgttatcttcgtcactatgaacatcacgcgtttaaaaccattgctaaatgctttggggaaatcacggtctttaaaggattcactctcgagcaacaaggtgaaatcatgcactccaagtggaagaaatatgttaatcccgttgcggtcggtctcgatgccagtcgattcgatcaacacgtgtctagggaagcacttgagtacgagcatgaattttatttgagagattatcctaatgataaacagctaaaatggttgcttaagcaacaattgagtaatgtaggcacagcattcgctagcgacggaatcataaagtacaagaaagagggatgtagaatgagtggggacatgaacacaagtttgggaaactgcatattgatgtgcgccatggtctttgggctaaaagaacacttaggaatgaaattgtcattggctaacaatggggatgactgcgtcattgtctgtgagaaagcggatttattgaaattgacgagcagcatcgaaccatatttcagacagttcggattcaaaatggaagtggaaaagcctgtagacatctttgagcgcattgaattttgccaaacccaacctgtgttcgatggctcccaatacattatggttaggaaaccctccgttgtaacttccaaagatgtcactagcttaataccgtgccaaacacaatctcaatacgcagaatggctgcaagctgttggtgagtgcggtatgagcataaatggtggaatacctgtcatgcagaatttctacaccatgttgcaaactggcgtaaagcgcacaaaattcaccaagaccggcgagttccaggcgaatgggctagggtatcactctcgatttatgaacagggtggcccgaactccttcgcctgagacccgtttatccttttacttagcgtttggtatcacaccagacctccaggaagcattggaggtcttctatgataccagtacgcttgaattggatgatgtgatcccgactgatacctaccaagtgtcaggagagcatttaatcaatggattaccaaactgatatcaccgaagataacgtgagcataagcggtcgggccaggaggggcactggggacaagaaacacaatggttcgggaatgtctggcgtaaagcgtcatgcggtgagtgaaacagctcagaaatcgcagcaaggtactggcaatggcacaatgaccaacatagctgaagaacagaccattaccgtgacatacaactttaacttttgagttatggctgtgtgtcgctgctgtgatacttcaccaggtattacattattcccttactttgcaattctcatcctcatccttgcaatactagttgttggaactccaaaccagcaatatcatcattctcctagcatttacgagtacaagactcaacacatttcgatcgcaaaatagacatttactataacaccaaaacatgcctaagagaggacgagttggactcgctgaatcttttcaaagaaagacgaagcaacagaaacgggcagagtacgaagctgtaaaacgtgagcagctcgaacgtgcattcgcaaacaattccaaggtagccaatcctagatcttctgggctaagcttccgaccgttggtggcaccaatcgccgggtccgttgtttacagcagacctcgcgtgccacagatccgcacgaaccaaatgtcaactattgtggtaaacactgaattggtagccaacatcactttggctgctgctggagcattcagtttcaccgcccagccattgataccatcatttggatcttggttggccaacatagctgacttgtactcaaaatggagatggattaggtgttcagtcatatacatacctaaatgtcccaccaccactcaaggtagtgtggttatggcgattgtgtatgatgcgcaggacaccgtacctacgacacgaacgcaggtatcacagtgttatcaatccatcacatttccaccgtacgccgggtacggtggcgcctctgcgctaaatagctacagctctggaggggaatcgctagtgtctacacttgacaccaatcgcgttgataagaagtggtacagcacaataggcaatgctgccttcactgctctcacatctatcgacaagaaccagttctgtccagccacagctctcattgctggggacggcggacctgtgccttccacagctgtgggcgatgtatttatgcgatatgagattgagttcatcgaacgaatcaaccctaccattaacgtttgagtgttaactggcttaaaccctaagggtagatatgtgggcggtaagcaagagggatcctgggaaacaggcttcgacgggttgggggtggtgccccgaccgacgcatcacttgctgatacaaccattagacacctaagggcgggtctagccaggtctccacgccatgatcaattggaaacgattgtgaggggggtagtggaacccataccagattgaggggcctttgccccacccc

SEQ ID NO: 2 - DNA, 335 bp, Tomato Spotted Wilt Virus
  source 1..335: mol_type = genomic DNA
agttgatataaagtagtttcctattgactcgttgtgacagtctttaaggaaggagaaggagaagttgactagagagttctaaactcgagtcaagaaattcgacaaaaaaatagacgaagagtgacaaaggaaatccttaatagtcgaacgtccgaagttacttacggactctagatcgagattaccgggacaaatctccatattggtatgttgaaaacagaaatagtcgagacccacttagtggtttgagaaaacaggttcttatgtactgtgatggttttctttggggaaagaacataagaaccgatgtgtagtttacgtcgactgttgtcaaa

SEQ ID NO: 3 - DNA, 4014 bp, synthetic construct
  source 1..4014: mol_type = other DNA
agtatacataccaagtatacggaataggtgtgaacccttgctcagctaaagaggataaaatggagctcactaaccactgcaagcaaactgctgctgaaggatttgtaagctttctgaactggctttgtaacccatggagacgacaacgaacagtcaacgctgctgttaagttccaacaggctctcctctcaatagaggatactgaacacttcgaggacatcaacgaatgcctcgaggagtctgctggagcccaatcacagcgaactaaggttgtcgccgaaggggcatattctcccgtcaaaaccaatcgtacccgccgagtccgcaagcagaagaaggccaagtttgtcaagtacttggtcaatgaggctcgtgccgagtttggtctacccaaagccactgaggccaatcgacttatggtacaacacttcttgctcagaacgtgtaaggaatggggtgtggtcacctcccaatgtcataacaacgttgcacttgcgttaaacctagtgttcatcccaactgaagatgacctgctgtcccgagcactgatgaacacttacgccacgcgagctgctgtgaatggaatgaccaacacccaaggggaggggtggtggaacaaccgacttgggattggatcccaggttggactggccttccgggccaaataggggtgcctagagaggaggccagggttctccacgtccgtttcgcgtggagagcaccctgatctggtggtcaaaccatcaggacaccccgagaaacagcgccagttgctgcgctatagtggaattggcggccatttactaattggcatccacaacaactctctctccaatttgcgccggggcttaatggaaagagtattctacgtcgagggacccaatgggctccaagacgccccgaaacccgacaagggagccttcaactcccttgctaagttcagagatctctatacaaagaatagctggcgtcattcccctgtaaccaatgagcaatttttgatgaattactcgggcaggaagctaactatttacaaggatgcggtcgacagtttgtcgcgtcaaccgcttagcctaagagatgctcggctgaagacattcgttaaggcggaaaaattgaatctgagtaagaaaccagatccagcaccgagggtcattcagcctcggtcgccccgctataacgtatgtttgggtcgttatcttcgtcactatgaacatcacgcgtttaaaaccattgctaaatgctttggggaaatcacggtctttaaaggattcactctcgagcaacaaggtgaaatcatgcactccaagtggaagaaatatgttaatcccgttgcggtcggtctcgatgccagtcgattcgatcaacacgtgtctagggaagcacttgagtacgagcatgaattttatttgagagattatcctaatgataaacagctaaaatggttgcttaagcaacaattgagtaatgtaggcacagcattcgctagcgacggaatcataaagtacaagaaagagggatgtagaatgagtggggacatgaacacaagtttgggaaactgcatattgatgtgcgccatggtctttgggctaaaagaacacttaggaatgaaattgtcattggctaacaatggggatgactgcgtcattgtctgtgagaaagcggatttattgaaattgacgagcagcatcgaaccatatttcagacagttcggattcaaaatggaagtggaaaagcctgtagacatctttgagcgcattgaattttgccaaacccaacctgtgttcgatggctcccaatacattatggttaggaaaccctccgttgtaacttccaaagatgtcactagcttaataccgtgccaaacacaatctcaatacgcagaatggctgcaagctgttggtgagtgcggtatgagcataaatggtggaatacctgtcatgcagaatttctacaccatgttgcaaactggcgtaaagcgcacaaaattcaccaagaccggcgagttccaggcgaatgggctagggtatcactctcgatttatgaacagggtggcccgaactccttcgcctgagacccgtttatccttttacttagcgtttggtatcacaccagacctccaggaagcattggaggtcttctatgataccagtacgcttgaattggatgatgtgatcccgactgatacctaccaagtgtcaggagagcatttaatcaatggattaccaaactgatatcaccgaagataacgtgagcataagcggtcgggccaggaggggcactggggacaagaaacacaatggttcgggaatgtctggcgtaaagcgtcatgcggtgagtgaaacagctcagaaatcgcagcaaggtactggcaatggcacaatgaccaacatagctgaagaacagaccattaccgtgacatacaactttaacttttgagttatggctgtgtgtcgctgctgtgatacttcaccaggtattacattattcccttactttgcaattctcatcctcatccttgcaatactagttgttggaactccaaaccagcaatatcatcattctcctagcatttacgagtacaagactcaacacatttcgatcgcaaaatagacatttactataacaccaaaacatgcctaagagaggacgagttggactcgctgaatcttttcaaagaaagacgaagcaacagaaacgggcagagtacgaagctgtaaaacgtgagcagctcgaacgtgcattcgcaaacaattccaaggtagccaatcctagatcttctgggctaagcttccgaccgttggtggcaccaatcgccgggtccgttgtttacagcagacctcgcgtgccacagatccgcacgaaccaaatgtcaactattgtggtaaacactgaattggtagccaacatcactttggctgctgctggagcattcagtttcaccgcccagccattgataccatcatttggatcttggttggccaacatagctgacttgtactcaaaatggagatggattaggtgttcagtcatatacatacctaaatgtcccaccaccactcaaggtagtgtggttatggcgattgtgtatgatgcgcaggacaccgtacctacgacacgaacgcaggtatcacagtgttatcaatccatcacatttccaccgtacgccgggtacggtggcgcctctgcgctaaatagctacagctctggaggggaatcgctagtgtctacacttgacaccaatcgcgttgataagaagtggtacagcacaataggcaatgctgccttcactgctctcacatctatcgacaagaaccagttctgtccagccacagctctcattgctggggacggcggacctgtgccttccacagctgtgggcgatgtatttatgcgatatgagattgagttcatcgaacgaatcaaccctaccattaacgtttgagtgttagttgatataaagtagtttcctattgactcgttgtgacagtctttaaggaaggagaaggagaagttgactagagagttctaaactcgagtcaagaaattcgacaaaaaaatagacgaagagtgacaaaggaaatccttaatagtcgaacgtccgaagttacttacggactctagatcgagattaccgggacaaatctccatattggtatgttgaaaacagaaatagtcgagacccacttagtggtttgagaaaacaggttcttatgtactgtgatggttttctttggggaaagaacataagaaccgatgtgtagtttacgtcgactgttgtcaaaaactggcttaaaccctaagggtagatatgtgggcggtaagcaagagggatcctgggaaacaggcttcgacgggttgggggtggtgccccgaccgacgcatcacttgctgatacaaccattagacacctaagggcgggtctagccaggtctccacgccatgatcaattggaaacgattgtgaggggggtagtggaacccataccagattgaggggcctttgccccacccc